European Patent Specification EP 4 237 584 B1, published April 23, 2025. Title: GENERIC CARTRIDGE AND METHOD FOR MULTIPLEX NUCLEIC ACID DETECTION. Applicant: Biocartis NV. The sequence listing filed with the application follows.

SEQUENCE LISTING (88 sequences)

SEQ ID NO: 1 - DNA, 19 bp, synthetic DNA
aaaagatcaaagtgctggc

SEQ ID NO: 2 - DNA, 25 bp, synthetic DNA
gaattcaaaaagatcaaagtgcaga

SEQ ID NO: 3 - DNA, 24 bp, synthetic DNA
aattcaaaaagatcaaagtgcggt

SEQ ID NO: 4 - DNA, 23 bp, synthetic DNA
ctcttgaggatcttgaaggatga

SEQ ID NO: 5 - DNA, 22 bp, synthetic DNA
gctctcttgaggatcttgtaga

SEQ ID NO: 6 - DNA, 20 bp, synthetic DNA
ctcttgaggatcttgatggc

SEQ ID NO: 7 - DNA, 23 bp, synthetic DNA
ctcttgaggatcttgaagcatac

SEQ ID NO: 8 - DNA, 20 bp, synthetic DNA
ctcttgaggatcttgatggg

SEQ ID NO: 9 - DNA, 21 bp, synthetic DNA
tctcttgaggatcttgatggt

SEQ ID NO: 10 - DNA, 21 bp, synthetic DNA
attcccgtcgctatcaaaaca

SEQ ID NO: 11 - DNA, 20 bp, synthetic DNA
ccgtcgctatcaagacatct

SEQ ID NO: 12 - DNA, 22 bp, synthetic DNA
ccgtcgctatcaaggaatcgaa

SEQ ID NO: 13 - DNA, 20 bp, synthetic DNA
cgtcgctatcaaggaatctc

SEQ ID NO: 14 - DNA, 19 bp, synthetic DNA
tcgctatcaaggaaccaac

SEQ ID NO: 15 - DNA, 19 bp, synthetic DNA
cgtcgctatcaaggttccg

SEQ ID NO: 16 - DNA, 19 bp, synthetic DNA
ccgtcgctatcaaggcatc

SEQ ID NO: 17 - DNA, 20 bp, synthetic DNA
gtcgctatcaaggaaccgaa

SEQ ID NO: 18 - DNA, 21 bp, synthetic DNA
cgtcgctatcaaggaaccatc

SEQ ID NO: 19 - DNA, 19 bp, synthetic DNA
cgtcgctatcaaggaagca

SEQ ID NO: 20 - DNA, 21 bp, synthetic DNA
cgtcgctatcaaggagccaac

SEQ ID NO: 21 - DNA, 21 bp, synthetic DNA
cgtcgctatcaaggaatcatc

SEQ ID NO: 22 - DNA, 22 bp, synthetic DNA
tcccgtcgctatcaaaatatct

SEQ ID NO: 23 - DNA, 19 bp, synthetic DNA
tcccgtcgctatcaagtct

SEQ ID NO: 24 - DNA, 20 bp, synthetic DNA
gtcgctatcaaggaacagaa

SEQ ID NO: 25 - DNA, 19 bp, synthetic DNA
ccgtcgctatcaaggctcc

SEQ ID NO: 26 - DNA, 19 bp, synthetic DNA
cgtcgctatcaaggatccg

SEQ ID NO: 27 - DNA, 19 bp, synthetic DNA
gtcgctatcaaggagcaat

SEQ ID NO: 28 - DNA, 20 bp, synthetic DNA
gaagcctacgtgatgggcat

SEQ ID NO: 29 - DNA, 20 bp, synthetic DNA
ctccaggaagccttccagga

SEQ ID NO: 30 - DNA, 17 bp, synthetic DNA
ctcatgcccttcggctc

SEQ ID NO: 31 - DNA, 17 bp, synthetic DNA
gctcatgcccttcggca

SEQ ID NO: 32 - DNA, 23 bp, synthetic DNA
gtcaagatcacagattttggtcg

SEQ ID NO: 33 - DNA, 24 bp, synthetic DNA
gtcaagatcacagattttgggcgt

SEQ ID NO: 34 - DNA, 20 bp, synthetic DNA
gattttgggctggccaaaca

SEQ ID NO: 35 - DNA, 24 bp, synthetic DNA
taggtgattttggtctagcttcaa

SEQ ID NO: 36 - DNA, 23 bp, synthetic DNA
ggtgattttggtctagctagaga

SEQ ID NO: 37 - DNA, 21 bp, synthetic DNA
aacttgtggtagttggagctt

SEQ ID NO: 38 - DNA, 22 bp, synthetic DNA
aacttgtggtagttggaggtgt

SEQ ID NO: 39 - DNA, 22 bp, synthetic DNA
aacttgtggtagttggaggtga

SEQ ID NO: 40 - DNA, 22 bp, synthetic DNA
ggaagcatacgtgatggcatac

SEQ ID NO: 41 - DNA, 22 bp, synthetic DNA
ggaagcatacgtgatggcttac

SEQ ID NO: 42 - DNA, 20 bp, synthetic DNA
ggctggtgtgggctccccgg

SEQ ID NO: 43 - DNA, 26 bp, synthetic DNA
gaacctctaagtcaagagccatctgt

SEQ ID NO: 44 - DNA, 17 bp, synthetic DNA
gcctgtgccagggacct

SEQ ID NO: 45 - DNA, 20 bp, synthetic DNA
ccccacacagcaaagcagaa

SEQ ID NO: 46 - DNA, 19 bp, synthetic DNA
gtggaggtgaggcagatgc

SEQ ID NO: 47 - DNA, 23 bp, synthetic DNA
cacacaccagttgagcaggtact

SEQ ID NO: 48 - DNA, 20 bp, synthetic DNA
cttactttgcctccttctgc

SEQ ID NO: 49 - DNA, 23 bp, synthetic DNA
cacaaaatggatccagacaactg

SEQ ID NO: 50 - DNA, 25 bp, synthetic DNA
catattcgtccacaaaatgattctg

SEQ ID NO: 51 - DNA, 18 bp, synthetic DNA
gctgcaccgtggatgtca

SEQ ID NO: 52 - DNA, 23 bp, synthetic DNA
gacatacctggaaaaatggaacc

SEQ ID NO: 53 - DNA, 44 bp, synthetic DNA
ccgatctacgtcgagcgcgttcggcacggtgtataaggtaaggt

SEQ ID NO: 54 - DNA, 45 bp, synthetic DNA
gcgagtcttacgctcggacaaggaaatcctcgatgtgagtttctg

SEQ ID NO: 55 - DNA, 39 bp, synthetic DNA
gtagatgcatagcctaccggacaacccccacgtgtgccg

SEQ ID NO: 56 - DNA, 46 bp, synthetic DNA
tggggagttactgtaccgatggactatgtccgggaacacaaagaca

SEQ ID NO: 57 - DNA, 46 bp, synthetic DNA
gcaacatcagatatcgcgtgcggaagagaaagaataccatgcagaa

SEQ ID NO: 58 - DNA, 45 bp, synthetic DNA
cgagctaactacggtacgtctcgatggagtgggtcccatcagttt

SEQ ID NO: 59 - DNA, 43 bp, synthetic DNA
gtgtcactcgattacgcgcaagagtgccttgacgatacagcta

SEQ ID NO: 60 - DNA, 41 bp, synthetic DNA
cggaggactgtcgcgtatatgcccagaaggcgggagacata

SEQ ID NO: 61 - DNA, 44 bp, synthetic DNA
gtactgagtcgccgaatctggtgtggattgttcatcaattggcg

SEQ ID NO: 62 - DNA, 80 bp, synthetic DNA
actagtcatcgcgtaatcgccggggccccttttttggggccccggccagtaaaaataggtgattttggtctagctagaga

SEQ ID NO: 63 - DNA, 70 bp, synthetic DNA
cgtgtctgaagcgcgcgaggggccccttttttggggcccctcgaccaagctctcttgaggatcttgatga

SEQ ID NO: 64 - DNA, 67 bp, synthetic DNA
gctatctgtacgcgattcgacggggccccttttggggccccgtccaggaagcctacgtgatggcgat

SEQ ID NO: 65 - DNA, 64 bp, synthetic DNA
tcgttctgggctctacgacggggccccttttggggccccgtccagattttgggctggccaatca

SEQ ID NO: 66 - DNA, 72 bp, synthetic DNA
actagtcatcgcgtaatcgccggggccccttttttggggccccggcataggtgattttggtctagctacaga

SEQ ID NO: 67 - DNA, 39 bp, synthetic DNA
gtgtcactcgattacgcgctccaactaccgacgtatcgg

SEQ ID NO: 68 - DNA, 52 bp, synthetic DNA
gctgaaaatgactgaatataaacttaccccgatacgtcggtagttggagctt

SEQ ID NO: 69 - DNA, 19 bp, synthetic DNA
cgggaagtcagacgggtca

SEQ ID NO: 70 - DNA, 20 bp, synthetic DNA
gagaggtaccggcaggagca

SEQ ID NO: 71 - DNA, 24 bp, synthetic DNA
ggaagcccaggataaaatgtggct

SEQ ID NO: 72 - DNA, 22 bp, synthetic DNA
aagtgcctcagggaccccttca

SEQ ID NO: 73 - DNA, 25 bp, synthetic DNA
gccatagtctcttccctagccccat

SEQ ID NO: 74 - DNA, 24 bp, synthetic DNA
gccaattaccaatgacccctcctt

SEQ ID NO: 75 - DNA, 26 bp, synthetic DNA
gaacctctaagtcaagagccatctgt

SEQ ID NO: 76 - DNA, 23 bp, synthetic DNA
gacatacctggaaaaatggaacc

SEQ ID NO: 77 - DNA, 21 bp, synthetic DNA
gccgttctggagctgttgata

SEQ ID NO: 78 - DNA, 24 bp, synthetic DNA
gagagatgcaggagaaattgttgc

SEQ ID NO: 79 - DNA, 22 bp, synthetic DNA
tctaagtcaagagccatctgta

SEQ ID NO: 80 - DNA, 26 bp, synthetic DNA
gatatgacatacctggaaaaatggaa

SEQ ID NO: 81 - DNA, 22 bp, synthetic DNA
ccccagaccccggctgcagcgc

SEQ ID NO: 82 - DNA, 32 bp, synthetic DNA
ctaaggaggtaagcctcagagcgtcccattcc

SEQ ID NO: 83 - DNA, 27 bp, synthetic DNA
cgtgacccacataccctgacccacccc

SEQ ID NO: 84 - DNA, 45 bp, synthetic DNA
actgagtcgccgaatcgctggtgtggattgttcatcaattggcgg

SEQ ID NO: 85 - DNA, 48 bp, synthetic DNA
ctcgtctgcttgtacactgactcgggaagctggaaatataaatcaatc

SEQ ID NO: 86 - DNA, 25 bp, synthetic DNA
accccgccaattgatgaacaatcca

SEQ ID NO: 87 - DNA, 51 bp, synthetic DNA
cagccggccaagacgcgccggcttggcgattcggcgactcagtactatcag

SEQ ID NO: 88 - DNA, 50 bp, synthetic DNA
cagccggccaagacgcgccggcttgggatcagtgtacaagcagacgagaa